European Patent Application EP 4 491 192 A1, published January 15, 2025. Title: Antibody-Drug Conjugates or CAR-T cells for the treatment and/or prevention of Leukemia. Applicant: Consejo Superior de Investigaciones Cientificas (CSIC). The sequence listing filed with the application follows.

SEQUENCE LISTING (12 sequences)

SEQ ID NO: 1 - protein, 5 aa, synthetic construct
RYAMS

SEQ ID NO: 2 - protein, 18 aa, synthetic construct
AAISSGGSYTYYPDSVKG

SEQ ID NO: 3 - protein, 13 aa, synthetic construct
LRVVAEGGSYFDY

SEQ ID NO: 4 - protein, 16 aa, synthetic construct
RSSQSILHSNGNTYLE

SEQ ID NO: 5 - protein, 7 aa, synthetic construct
KVSNRFS

SEQ ID NO: 6 - protein, 9 aa, synthetic construct
FQGSHVPVT

SEQ ID NO: 7 - protein, 122 aa, synthetic construct
EVQLVESGGGLVKPGGSLQLSCAASGFTFNRYAMSWVRQTPEKRLEWVAAISSGGSYTYYPDSVKGRFIISRDNAKNTLSLQMSSLRSEDTAMFYCARLRVVAEGGSYFDYWGQGTTLTVSS

SEQ ID NO: 8 - protein, 112 aa, synthetic construct
DVLMTQTPLSLPVSLGDQASISCRSSQSILHSNGNTYLEWYLQKPGQSPKLLIYKVSNRFSGVPDRFSGSGSGTDFTLKISRVEAEDLGVYYCFQGSHVPVTFGSGTKLEIK

SEQ ID NO: 9 - DNA, 366 bp, synthetic construct
  source 1..366: mol_type = other DNA
gaagtgcagttggtggagtctgggggaggcttagtgaagcctggagggtccctgcaactctcctgtgcagcctctggattcactttcaatagatatgccatgtcttgggttcgccagactccggagaagaggctggagtgggtcgcagccattagtagtggtggtagttacacctactatccagacagtgtgaagggtcgattcatcatctccagagacaatgccaagaacaccctgtccctgcaaatgagcagtctgaggtctgaggacacggccatgttttactgtgcaagactcagggtagtagctgaagggggtagctactttgactactggggccaaggcaccactctcacagtctcctca

SEQ ID NO: 10 - DNA, 336 bp, synthetic construct
  source 1..336: mol_type = other DNA
gatgttttgatgacccaaactccactctccctgcctgtcagtcttggagatcaagcctccatctcttgcagatctagtcagagcattttacatagtaatggaaacacctatttagaatggtacctgcagaaaccaggccagtctccaaagctcctgatctacaaagtttccaaccgattttctggggtcccagacaggttcagtggcagtggatcagggacagatttcacactcaagatcagcagagtggaggctgaggatctgggagtttattactgctttcaaggttcacatgttcctgtcacgttcggctcggggacaaagttagaaataaaa

SEQ ID NO: 11 - DNA, 846 bp, synthetic construct
  source 1..846: mol_type = other DNA
gccaccatgggatggtcctgtatcattctgttcctggtcgcaactgccaccggggtccactccgaagtccagctggtcgagagcgggggcggcctggtgaagccaggaggctccctgcagctgtcttgcgccgccagcggcttcacctttaaccggtacgccatgtcttgggtgcggcagacacctgagaagagactggagtgggtggcagcaatcagctccggaggctcttatacctactatccagacagcgtgaagggcaggttcatcatctcccgcgataacgccaagaataccctgtccctgcagatgtctagcctgagatctgaggacacagccatgttctactgcgcaaggctgagagtggtggcagagggaggcagctactttgattattggggccagggcaccacactgaccgtgtcctctggcggcggcggctccggaggcggcggctctggaggaggaggcagcggcggaggaggctccgacgtgctgatgacccagacaccactgtccctgcccgtgagcctgggcgatcaggcctctatcagctgtaggagctcccagagcatcctgcactccaacggcaatacatacctggagtggtatctgcagaagccaggccagtcccccaagctgctgatctataaggtgtctaataggttcagcggcgtgcctgaccgcttttccggctctggcagcggcaccgatttcacactgaagatcagcagggtggaggcagaggacctgggcgtgtactattgttttcagggctcccacgtgcctgtcaccttcggctctggaactaaactggaaatcaaacatcaccaccatcaccactaa

SEQ ID NO: 12 - protein, 281 aa, synthetic construct
ATMGWSCIILFLVATATGVHSEVQLVESGGGLVKPGGSLQLSCAASGFTFNRYAMSWVRQTPEKRLEWVAAISSGGSYTYYPDSVKGRFIISRDNAKNTLSLQMSSLRSEDTAMFYCARLRVVAEGGSYFDYWGQGTTLTVSSGGGGSGGGGSGGGGSGGGGSDVLMTQTPLSLPVSLGDQASISCRSSQSILHSNGNTYLEWYLQKPGQSPKLLIYKVSNRFSGVPDRFSGSGSGTDFTLKISRVEAEDLGVYYCFQGSHVPVTFGSGTKLEIKHHHHHH